European Patent Specification EP 3 986 412 B1, published September 30, 2026. Title: AGENTS FOR REVERSING TOXIC PROTEINOPATHIES. Applicant: THE BROAD INSTITUTE, INC. THE BRIGHAM & WOMEN'S HOSPITAL, INC. DANA-FARBER CANCER INSTITUTE, INC. The sequence listing filed with the application follows.

SEQUENCE LISTING (13 sequences)

SEQ ID NO: 1 - DNA, 3607 bp, Homo sapiens
atgacaccgggcacccagtctcctttcttcctgctgctgctcctcacagtgcttacagttgttacgggttctggtcatgcaagctctaccccaggtggagaaaaggagacttcggctacccagagaagttcagtgcccagctctactgagaagaatgctgtgagtatgaccagcagcgtactctccagccacagccccggttcaggctcctccaccactcagggacaggatgtcactctggccccggccacggaaccagcttcaggttcagctgccacctggggacaggatgtcacctcggtcccagtcaccaggccagccctgggctccaccaccccaccagcccacgatgtcacctcagccccggacaacaagccagccccgggctccaccgccccccccagcccacggtgtcacctcggccccggacaccaggccggccccgggctccaccgccccccaagcccacggtgtcacctcggccccggacaccaggccggccccgggctccaccgcccccccagcccacggtgtcacctcggccccggacaccaggcccgccccgggctccaccgcccccccagcccacggtgtcacctcggccccggacaccaggccggccccgggctccaccgcccccccagcccacggtgtcacctcggccccggagagcaggccggccccgggctccaccgcgcccgcagcccacggtgtcacctcggccccggagagcaggccggccccgggctccaccgcgcccgcagcccacggtgtcacctcggccccggagagcaggccggccccgggctccaccgcgcccgcagcccacggtgtcacctcggccccggagagcaggccggccccgggctccaccgcgcccgcagcccacggtgtcacctcggccccggagagcaggccggccccgggctccaccgcccccccagcccacggtgtcacctcggccccggacaccaggccggccccgggctccaccgcccccccagcccacggtgtcacctcggccccggacaccaggccggccccgggctccaccgcccccccagcccacggtgtcacctcggccccggacaccaggccggccccgggctccaccgcccccccagcccacggtgtcacctcggccccggacaccaggccggccccgggctccaccgcccccccagcccacggtgtcacctcggccccggagagcaggccggccccgggctccaccgcccccccagcccacggtgtcacctcggccccggagagcaggccggccccgggctccaccgcgcccgcagcccacggtgtcacctcggccccggagagcaggccggccccgggctccaccgcgcccgcagcccacggtgtcacctcggccccggagagcaggccggccccgggctccaccgcccccccagcccacggtgtcacctcggccccggacaccaggccggccccgggctccaccgcccccccagcccacggtgtcacctcggccccggacaccaggccggccccgggctccaccgcccccccagcccacggtgtcacctcggccccggacaccaggccggccccgggctccaccgcccccccagcccacggtgtcacctcggccccggacaccaggccggccccgggctccaccgcccccccagcccacggtgtcacctcggccccggacaccaggccggccccgggctccaccgcccccccagcccacggtgtcacctcggccccggacaccaggccggccccgggctccaccgcccccccagcccacggtgtcacctcggccccggacaccaggccggccccgggctccaccgcccccccagcccacggtgtcacctcggccccggacaccaggccggccccgggctccaccgcgcccgcagcccacggtgtcacctcggccccggagagcaggccggccccgggctccaccgcgcccgcagcccacggtgtcacctcggccccggagagcaggccggccccgggctccaccgcccccccagcccacggtgtcacctcggccccggacaccaggccggccccgggctccaccgcccccccagcccacggtgtcacctcggccccggacaccaggccggccccgggctccaccgcccccccagcccacggtgtcacctcggccccggacaccaggccggccccgggctccaccgcccccccagcccacggtgtcacctcggccccggacaccaggccggccccgggctccaccgcccccccagcccacggtgtcacctcggccccggacaccaggccggccccgggctccaccgcccccccagcccacggtgtcacctcggccccggacaccaggccggccccgggctccaccgcccccccagcccacggtgtcacctcggccccggacaccaggccggccccgggctccaccgcccccccagcccacggtgtcacctcggccccggacaccaggccggccccgggctccaccgcccccccagcccacggtgtcacctcggccccggacaccaggcgggccccgggctccaccccggccccgggctccaccgcccccccagcccacggtgtcaccttggccccggacaccaggccggccccgggctccaccgcccccccagcccatggtgtcacctcggccccggacaacaggcccgccttgggctccaccgcccctccagtccacaatgtcacctcggcctcaggctctgcatcaggctcagcttctactctggtgcacaacggcacctctgccagggctaccacaaccccagccagcaagagcactccattctcaattcccagccaccactctgatactcctaccacccttgccagccatagcaccaagactgatgccagtagcactcaccatagctcggtacctcctctcacctcctccaatcacagcacttctccccagttgtctactggggtctctttctttttcctgtcttttcacatttcaaacctccagtttaattcctctctggaagatcccagcaccgactactaccaagagctgcagagagacatttctgaaatgtttttgcagatttataaacaagggggttttctgggcctctccaatattaagttcaggccaggatctgtggtggtacaattgactctggccttccgagaaggtaccatcaatgtgcacgacgtggagacacagttcaatcagtataaaacggaagcagcctctcgatataacctgacgatctcagacgtcagcgtgagtgatgtgccatttcctttctctgcccagtctggggctggggtgccaggctggggcatcgcgctgctggtgctggtctgtgttctggttgcgctggccattgtctatctcattgccttggctgtctgtcagtgccgccgaaagaactacgggcagctggacatctttccagcccgggatacctaccatcctatgagcgagtaccccacctaccacacccatgggcgctatgtgccccctagcagtaccgatcgtagcccctatgagaaggtttctgcaggtaacggtggcagcagcctctcttacacaaacccagcagtggcagccacttctgccaacttgtag

SEQ ID NO: 2 - DNA, 1923 bp, Homo sapiens
atggggcagccatctctgacttggatgctgatggtggtggtggcctcttggttcatcacaactgcagccactgacacctcagaagcaagatggtgctctgaatgtcacagcaatgccacctgcacggaggatgaggccgttacgacgtgcacctgtcaggagggcttcaccggcgatggcctgacctgcgtggacctggatgagtgcgccattcctggagctcacaactgctccgccaacagcagctgcgtaaacacgccaggctccttctcctgcgtctgccccgaaggcttccgcctgtcgcccggtctcggctgcacagacgtggatgagtgcgctgagcctgggcttagccactgccacgccctggccacacgtgtcaatgtggtgggcagctacttgtgcgtatgccccgcgggctaccggggggatggatggcactgtgagtgctccccgggctcctgcgggccggggttggactgcgtgcccgagggcgacgcgctcgtgtgcgcggatccgtgccaggcgcaccgcaccctggacgagtactggcgcagcaccgagtacggggagggctacgcctgcgacacggacctgcgcggctggtaccgcttcgtgggccagggcggtgcgcgcatggccgagacctgcgtgccagtcctgcgctgcaacacggccgcccccatgtggctcaatggcacgcatccgtccagcgacgagggcatcgtgagccgcaaggcctgcgcgcactggagcggccactgctgcctgtgggatgcgtccgtccaggtgaaggcctgtgccggcggctactacgtctacaacctgacagcgccccccgagtgtcacctggcgtactgcacagaccccagctccgtggaggggacgtgtgaggagtgcagtatagacgaggactgcaaatcgaataatggcagatggcactgccagtgcaaacaggacttcaacatcactgatatctccctcctggagcacaggctggaatgtggggccaatgacatgaaggtgtcgctgggcaagtgccagctgaagagtctgggcttcgacaaggtcttcatgtacctgagtgacagccggtgctcgggcttcaatgacagagacaaccgggactgggtgtctgtagtgaccccagcccgggatggcccctgtgggacagtgttgacgaggaatgaaacccatgccacttacagcaacaccctctacctggcagatgagatcatcatccgtgacctcaacatcaaaatcaactttgcatgctcctaccccctggacatgaaagtcagcctgaagaccgccctacagccaatggtcagtgctctaaacatcagagtgggcgggaccggcatgttcaccgtgcggatggcgctcttccagaccccttcctacacgcagccctaccaaggctcctccgtgacactgtccactgaggcttttctctacgtgggcaccatgttggatgggggcgacctgtcccgatttgcactgctcatgaccaactgctatgccacacccagtagcaatgccacggaccccctgaagtacttcatcatccaggacagatgcccacacactagagactcaactatccaagtggtggagaatggggagtcctcccagggccgattttccgtccagatgttccggtttgctggaaactatgacctagtctacctgcactgtgaagtctatctctgtgacaccatgaatgaaaagtgcaagcctacctgctctgggaccagattccgaagtgggagtgtcatagatcaatcccgtgtcctgaacttgggtcccatcacacggaaaggtgtccaggccacagtctcaagggcttttagcagcttggggctcctgaaagtctggctgcctctgcttctctcggccaccttgaccctgacttttcagtga

SEQ ID NO: 3 - DNA, 2768 bp, Homo sapiens
agagtcatccagctggagccctgagtggctgagctcaggccttcgcagcattcttgggtgggagcagccacgggtcagccacaagggccacagccatgaatggcacagaaggccctaacttctacgtgcccttctccaatgcgacgggtgtggtacgcagccacttcgagtacccacagtactacctggctgagccatggcagttctccatgctggccgcctacatgtttctgctgatcgtgctgggcttccccatcaacttcctcacgctctacgtcaccgtccagcacaagaagctgcgcacgcctctcaactacatcctgctcaacctagccgtggctgacctcttcatggtcctaggtggcttcaccagcaccctctacacctctctgcatggatacttcgtcttcgggcccacaggatgcaatttggagggcttctttgccaccctgggcggtgaaattgccctgtggtccttggtggtcctggccatcgagcggtacgtggtggtgtgtaagcccatgagcaacttccgcttcggggagaaccatgccatcatgggcgttgccttcacctgggtcatggcgctggcctgcgccgcacccccactcgccggctggtccaggtacatccccgagggcctgcagtgctcgtgtggaatcgactactacacgctcaagccggaggtcaacaacgagtcttttgtcatctacatgttcgtggtccacttcaccatccccatgattatcatctttttctgctatgggcagctcgtcttcaccgtcaaggaggccgctgcccagcagcaggagtcagccaccacacagaaggcagagaaggaggtcacccgcatggtcatcatcatggtcatcgctttcctgatctgctgggtgccctacgccagcgtggcattctacatcttcacccaccagggctccaacttcggtcccatcttcatgaccatcccagcgttctttgccaagagcgccgccatctacaaccctgtcatctatatcatgatgaacaagcagttccggaactgcatgctcaccaccatctgctgcggcaagaacccactgggtgacgatgaggcctctgctaccgtgtccaagacggagacgagccaggtggccccggcctaagacctgcctaggactctgtggccgactataggcgtctcccatcccctacaccttcccccagccacagccatcccaccaggagcagcgcctgtgcagaatgaacgaagtcacataggctccttaattttttttttttttttaagaaataattaatgaggctcctcactcacctgggacagcctgagaagggacatccaccaagacctactgatctggagtcccacgttccccaaggccagcgggatgtgtgcccctcctcctcccaactcatctttcaggaacacgaggattcttgctttctggaaaagtgtcccagcttagggataagtgtctagcacagaatggggcacacagtaggtgcttaataaatgctggatggatgcaggaaggaatggaggaatgaatgggaagggagaacatatctatcctctcagaccctcgcagcagcagcaactcatacttggctaatgatatggagcagttgtttttccctccctgggcctcactttcttctcctataaaatggaaatcccagatccctggtcctgccgacacgcagctactgagaagaccaaaagaggtgtgtgtgtgtctatgtgtgtgtttcagcactttgtaaatagcaagaagctgtacagattctagttaatgttgtgaataacatcaattaatgtaactagttaattactatgattatcacctcctgatagtgaacattttgagattgggcattcagatgatggggtttcacccaaccttggggcaggtttttaaaaattagctaggcatcaaggccagaccagggctgggggttgggctgtaggcagggacagtcacaggaatgcagaatgcagtcatcagacctgaaaaaacaacactgggggagggggacggtgaaggccaagttcccaatgagggtgagattgggcctggggtctcacccctagtgtggggccccaggtcccgtgcctccccttcccaatgtggcctatggagagacaggcctttctctcagcctctggaagccacctgctcttttgctctagcacctgggtcccagcatctagagcatggagcctctagaagccatgctcacccgcccacatttaattaacagctgagtccctgatgtcatccttatctcgaagagcttagaaacaaagagtgggaaattccactgggcctaccttccttggggatgttcatgggccccagtttccagtttcccttgccagacaagcccatcttcagcagttgctagtccattctccattctggagaatctgctccaaaaagctggccacatctctgaggtgtcagaattaagctgcctcagtaactgctcccccttctccatataagcaaagccagaagctctagctttacccagctctgcctggagactaaggcaaattgggccattaaaagctcagctcctatgttggtattaacggtggtgggttttgttgctttcacactctatccacaggatagattgaaactgccagcttccacctgatccctgaccctgggatggctggattgagcaatgagcagagccaagcagcacagagtcccctggggctagaggtggaggaggcagtcctgggaatgggaaaaacccca

SEQ ID NO: 4 - DNA, 2546 bp, Homo sapiens
aggtggagcaagatggctgtggagctgggcgtgctgctcgtccggccccggcccggaaccgggctgggtagagtgatgcggaccctcctgctggtgctgtggctggcgacgcgcggaagcgcgctctactttcacatcggagagacggagaagaagtgctttattgaggagatcccggacgagaccatggtcataggaaactaccggacgcagctgtatgacaagcagcgggaggagtaccagccggccaccccggggcttggcatgtttgtggaggtgaaggacccagaggacaaggtcatcctggcccggcagtatggctccgagggcaggttcactttcacttcccatacccctggtgagcaccagatctgtcttcactccaattccaccaagttctccctctttgctggaggcatgctgagagttcacctggacatccaggtaggtgaacatgccaatgactatgcagaaattgctgctaaagacaagttgagtgagttgcagctacgagtgcgacagctggtggaacaagtggagcagatccagaaagagcagaactaccagcggtggcgagaggagcgcttccggcagaccagtgagagcaccaaccagcgggtgctgtggtggtccattctgcagaccctcatcctcgtggccatcggtgtctggcagatgcggcacctcaagagcttctttgaagccaagaagcttgtgtagctgtcccaggcgtcacaacccatcctcccaggctgggggagaaaggacctcctggaactgacttcttctgtcaggaggactggtttccagccatacctgttctggaagggagaggggctggaggcacccacaggcacaagctgaaggcagcagcttggctaatactgagcaggtagtggggcaaattcctgccctctctctctggcctctgggccgtttggtagtaatcacccaagggctggtaaagcccctcctcttggcacctcagaatcacagtgttactgatcagggatgtgaggctgctgttgggggtggggggaggggaatgggcaggcaagccagtcttctgtcttcctttgctaacttagggttttgagcaggttggggtatggtgcctgtcatacccacctgccaccctgggaacctcactgttctctctttcagcctagacctgctgatccagggtgtgtgtgagttgagggtgggtggaggggtttgcagtgtgggaatgtggccctgcagttgacctgagctgcttcacatggttgtccattctggggcttaaagaactgggaccagaccaagtagaggccttggtgctggttggggtggggcctgcagagtcttagttactgatttcattttcaataaatgtaggtttgttacatgagtttcccaataaaaaaaaaaatgacttcttgtccagtgcaagtgactcagtcatcagtgggcacacactgcagggtgcctcagggaatgccagttcttccaaagagcaaagcacttcacattccaaagtgaattcccaccagtcagcttcattctttccttcttctccaggccttcctgtggcagggaatagtgggtttgtccaagattatacaacaagtaaattgggctggggctcaaatttacaccctttcctctgtgccagctccctggtgaagttccctctttctagagtcagtaagcaggattgtcatggatgctgccaggaagtgcctggtaaggaggtgcattgagcaggggagtgctacaggacagccaccctgggctggcagggacaaggatgttgatgggctaaaccaacagcaagtgatttcaaccaggaccatgaaggagaggaaggattctgctggaaggagatggcaggacaggggtggttggagaagtggaggcaaacagctggaatggaggtgggtgggtgtttaatttcagctgcagagggtgttgtgaggaagctggaaaggaaggttggattagagaagcctcgagctccaggtaagcgatttggacatgcccacctttcaagaggggctgcaggcacccacaggcacaagctgaaggcagcagcttggctggcttaatactgagcaggtggtggggtaaatgcctgcccccctccctctggcctctgggccctttgcagtaatcacccagggtctggtaaagccactgagagccctactggcacctcagaatcacagtgttattgatcagggatgtgaggctgctgttgggggttgggggaggcaaatgggcaggcagttttgagaagaaccttctaataagaaatgtgagggaggttacagcagtgtgtgagaaagaccaggaagaaggagacaagtttgggggctgcttcccctaatgggatgatgcaatctgggctcatgctgccaactaattcttccacatgaaaaaaaaaagttttttggcgggcacggtggttcacacctgtaatcccagcactttgggaggctgaggtaggtggatggcctgaggccaggagtttgagaccagcctggccaacatggtgaaacctcatc

SEQ ID NO: 5 - protein, 235 aa, Homo sapiens
MAVELGVLLVRPRPGTGLGRVMRTLLLVLWLATRGSALYFHIGETEKKCFIEEIPDETMVIGNYRTQLYDKQREEYQPATPGLGMFVEVKDPEDKVILARQYGSEGRFTFTSHTPGEHQICLHSNSTKFSLFAGGMLRVHLDIQVGEHANDYAEIAAKDKLSELQLRVRQLVEQVEQIQKEQNYQRWREERFRQTSESTNQRVLWWSILQTLILVAIGVWQMRHLKSFFEAKKLV

SEQ ID NO: 6 - DNA, 27 bp, Artificial
  synthetic
ggcagagaaaggaaatggcacatcact

SEQ ID NO: 7 - DNA, 27 bp, Artificial
  synthetic
ctgctgctcctcacagtgcttacaggt

SEQ ID NO: 8 - DNA, 20 bp, Artificial
  synthetic
gctaccacagcccctaaacc

SEQ ID NO: 9 - DNA, 19 bp, Artificial
  synthetic
gctgtggctggagagtacg

SEQ ID NO: 10 - DNA, 20 bp, Artificial
  synthetic
ccagccatagcaccaagact

SEQ ID NO: 11 - DNA, 20 bp, Artificial
  synthetic
ggaaggaaaggccgatactc

SEQ ID NO: 12 - DNA, 22 bp, Artificial
  synthetic
ttacgagagaaaactcatggcc

SEQ ID NO: 13 - DNA, 22 bp, Artificial
  synthetic
gggtccaagttgtccagaatgc